European Patent Specification EP 3 622 080 B1, published March 27, 2024. Title: Improved methods for producing isobutene from 3-methylcrotonic acid. Applicant: Global Bioenergies. The sequence listing filed with the application follows.

SEQUENCE LISTING (71 sequences)

SEQ ID NO: 1 - protein, 229 aa, Candida albicans
  Candida albicans (strain SC5314 / ATCC MYA-2876)
MIARVCLRRSNVLPIFQIPSRKYSINYEKVNNSIYNNVIKPKRIVLAITGATGTQIGVRLLEILKELGVETHLVMSKWGIATLKYETDYQVDYVTSLATKTYSARDVTAPISSGSFVHDGMIVAPCSMKSLSAIRTGFTEDLIVRAADVSLKERRKLLLVARETPLSDIHLDNMLYLSRMGVTIFPPVPAFYTKPKTIDDIVEQTCGRILDNFGINIDTFERWDGINHR

SEQ ID NO: 2 - protein, 227 aa, Aspergillus niger
MFNSLLSGTTTPNSGRASPPASEMPIDNDHVAVARPAPRRRRIVVAMTGATGAMLGIKVLIALRRLNVETHLVMSKWAEATIKYETDYHPSNVRALADYVHNINDMAAPVSSGSFRADGMIVVPCSMKTLAAIHSGFCDDLISRTADVMLKERRRLVLVARETPLSEIHLRNMLEVTRAGAVIFPPVPAFYIKAGSIEDLIDQSVGRMLDLFDLDTGDFERWNGWEK

SEQ ID NO: 3 - protein, 242 aa, Saccharomyces cerevisiae S288c
MLLFPRRTNIAFFKTTGIFANFPLLGRTITTSPSFLTHKLSKEVTRASTSPPRPKRIVVAITGATGVALGIRLLQVLKELSVETHLVISKWGAATMKYETDWEPHDVAALATKTYSVRDVSACISSGSFQHDGMIVVPCSMKSLAAIRIGFTEDLITRAADVSIKENRKLLLVTRETPLSSIHLENMLSLCRAGVIIFPPVPAFYTRPKSLHDLLEQSVGRILDCFGIHADTFPRWEGIKSK

SEQ ID NO: 4 - protein, 180 aa, Cryptococcus gattii WM276
  serotype B
MRRKRYVVAVTGATGATLAIRLLQALRALDIETHLIISKWAVKTLKYETDMIERELKDLADYSYSNSDLAAPPSSGSFIHDGMFIIPCSMKTLAAVRIGLGDELISRSADVCLKEGRKLMLVVRETPLNDIHLENMLFLRRAGAIIFPPVPAYYIRPQTIDDLTNQTVGRILDSSKCSQK

SEQ ID NO: 5 - protein, 189 aa, Escherichia coli K-12
MKRLIVGISGASGAIYGVRLLQVLRDVTDIETHLVMSQAARQTLSLETDFSLREVQALADVTHDARDIAASISSGSFQTLGMVILPCSIKTLSGIVHSYTDGLLTRAADVVLKERRPLVLCVRETPLHLGHLRLMTQAAEIGAVIMPPVPAFYHRPQSLDDVINQTVNRVLDQFAITLPEDLFARWQGA

SEQ ID NO: 6 - protein, 192 aa, Bacillus subtilis
MKLVIGMTGATGAIFGIRLLEYLKAAEIETHLVVSPWANVTITHETDYTLKDVEKLASYTYSHKDQAAAISSGSFETDGMIIAPCSMKSLASIRTGMADNLLTRAADVILKERKKLVLLTRETPLSQIHLENMLALTKMGSVILPPMPAFYNKPADMDELIDHIVFRTLDQFGIRLPEAKRWYGIEKQKGGI

SEQ ID NO: 7 - protein, 209 aa, Pseudomonas aeruginosa
MSGPERITLAMTGASGAQYGLRLLDCLVQEEREVHFLISKAAQLVMATETDVALPAKPQAMQAFLTEYCGAAAGQIRVFGQNDWMAPPASGSSAPNAMVICPCSTGTLSAVATGACNNLIERAADVALKERRPLVLVPREAPFSSIHLENMLKLSNLGAVILPAAPGFYHQPQSVEDLVDFVVARILNTLGIPQDMLPRWGEQHLVSDE

SEQ ID NO: 8 - protein, 219 aa, Enterobacter sp.
  Enterobacter sp. DC4
MLRQVRANALTCNSPQNPAQSALKSVRAKIMKRLIVGLSGASGAIYGVRLLQVLRNVAEVETHLVMSQAARQTLSLETDLSLRDVQALADVVHDARDIAASISSGSFKTAGMVILPCSIKTLSGIVNSYTDTLVTRAADVVLKERRPLVLCVRETPLHLGHLRLMTQAAELGAIIMPPVPAFYHRPTSLDDVINQTVNRVLDQFDIDLPEDLFTRWQGA

SEQ ID NO: 9 - protein, 503 aa, Saccharomyces cerevisiae S288c
MRKLNPALEFRDFIQVLKDEDDLIEITEEIDPNLEVGAIMRKAYESHLPAPLFKNLKGASKDLFSILGCPAGLRSKEKGDHGRIAHHLGLDPKTTIKEIIDYLLECKEKEPLPPITVPVSSAPCKTHILSEEKIHLQSLPTPYLHVSDGGKYLQTYGMWILQTPDKKWTNWSIARGMVVDDKHITGLVIKPQHIRQIADSWAAIGKANEIPFALCFGVPPAAILVSSMPIPEGVSESDYVGAILGESVPVVKCETNDLMVPATSEMVFEGTLSLTDTHLEGPFGEMHGYVFKSQGHPCPLYTVKAMSYRDNAILPVSNPGLCTDETHTLIGSLVATEAKELAIESGLPILDAFMPYEAQALWLILKVDLKGLQALKTTPEEFCKKVGDIYFRTKVGFIVHEIILVADDIDIFNFKEVIWAYVTRHTPVADQMAFDDVTSFPLAPFVSQSSRSKTMKGGKCVTNCIFRQQYERSFDYITCNFEKGYPKGLVDKVNENWKRYGYK

SEQ ID NO: 10 - protein, 168 aa, Enterobacter sp.
  Enterobacter sp. MGH 24
MSTFDKHDLSGFVGKHLVYTYDNGWNYEIYVKNETTLDYRIHSGLVANRWVKDQQAYIVRVGESIYKISWTEPTGTDVSLIVNLGDKLFHGTIFFPRWVMNNPEKTVCFQNDHIPLMNSYRDAGPAYPTEVIDEFATITFVRDCGANNESVIACAASELPNDFPANLN

SEQ ID NO: 11 - protein, 161 aa, Bacillus pumilus
MDQFVGLHMIYTYENGWEYEIYIKNDHTIDYRIHSGMVGGRWVRDQEVNIVKLTKGVYKVSWTEPTGTDVSLNFMPEEKRMHGVIFFPKWVHERPDITVCYQNDYIDLMKESREKYETYPKYVVPEFADITYIHHAGVNDETIIAEAPYEGMTDEIRAGRK

SEQ ID NO: 12 - protein, 534 aa, Aspergillus niger CBS 513.88
MLRMLRPGRRIPTHPSRSFSTTPHRSNDSPALNFRSLLSALRAQDDLVDITQPASPDLEIAALTRRVYESHSPAPLFHNVTDTDPETGLFKILGAPVGLRADPATRFGRLAIQLGLPQNATPLDILEKLIAAKHSTPLPPTPVPASSAPCKENILHGSQIDMTKWPIPRLHPLDGGNYLATYGFHILQSPDKAWTSWSISRTMHVANTPRTIVAPIMPGQHIAQVHQMWADQGAKDTPWALVLGGPPAAAFVGGMPLPAFVSEDGYIGALCGEAMDVVKCETNDLYVPANAEIVLEGRISTTEKVGEGPMGEYHGYMFQDKAVPEPRIEVDCVTYRRDPVVPICVAGLAPDETHTVWGAAISAEILDALRGAELPVKMAWMPYEAQCCWVVVSVDVERLGRMGIKKEELSRRVGEVVFGTHAGWEAPKVFVVGDDVDVTDIGQFVWALATRYRPGADELVFEEADGLPMIPYMTRASRREVPNPGKGGKSVVNLLLPSEFEGKRPWVPGSFEGLYSEELKQKVLGRWGELFEKK

SEQ ID NO: 13 - protein, 513 aa, Candida dubliniensis CD36
MSLNPALKFRDFIQVLKNEGDLIEIDTEVDPNLEVGAITRKAYENKLAAPLFNNLKQDPENIDPKNLFRILGCPGGLRGFGNDHARIALHLGLDSQTPMKEIIDFLVANRNPKKYIPPVLVPNDQSPHKKHHLTKEQIDLTKLPVPLLHHGDGGKFIQTYGMWVLQTPDKSWTNWSIARGMVHDSKSITGLVINPQHVKQVSDAWVAAGKGDKIPFALCFGVPPAAILVSSMPIPDGATEAEYIGGLCNQAVPVVKCETNDLEVPADCEMVFEGYLDRDTLVREGPFGEMHGYCFPKDHHTQPLYRVNHISYRDQAIMPISNPGLCTDETHTLIGGLVSAETKYLISQHPVLSKIVEDVFTPYEAQALWLAVKINTHELVKLKTNAKELSNLVGDFLFRSKECYKVCSILHEIILVGDDIDIFDFKQLIWAYTTRHTPVQDQLYFDDVKPFALAPFASQGPLIKTRQGGKCVTTCIFPKQFTDPDFEFVTCNFNGYPEEVKNKISQNWDKYYK

SEQ ID NO: 14 - protein, 502 aa, Klebsiella pneumoniae
MTAPIQDLRDAIALLQQHDNQYLETDHPVDPNAELAGVYRHIGAGGTVKRPTRIGPAMMFNNIKGYPHSRILVGMHASRQRAALLLGCEASQLALEVGKAVKKPVAPVVVPASSAPCQEQIFLADDPDFDLRTLLPAPTNTPIDAGPFFCLGLALASDPVDASLTDVTIHRLCVQGRDELSMFLAAGRHIEVFRQKAEAAGKPLPITINMGLDPAIYIGACFEAPTTPFGYNELGVAGALRQRPVELVQGVSVPEKAIARAEIVIEGELLPGVRVREDQHTNSGHAMPEFPGYCGGANPSLPVIKVKAVTMRNNAILQTLVGPGEEHTTLAGLPTEASIWNAVEAAIPGFLQNVYAHTAGGGKFLGILQVKKRQPADEGRQGQAALLALATYSELKNIILVDEDVDIFDSDDILWAMTTRMQGDVSITTIPGIRGHQLDPSQTPEYSPSIRGNGISCKTIFDCTVPWALKSHFERAPFADVDPRPFAPEYFARLEKNQGSAK

SEQ ID NO: 15 - protein, 510 aa, Leptolyngbya sp.
MLIDQEQAKTDHPLGWNVPDINDLRAAIAHLKKFKGQYIETDHPVDPIAELAGVYRYIGAGGTVMRPTRIGPAMTFNNVKGYPNSRVLVGMMASRERVSILLGAPTRELGMQMGKAVKTIVPPATIDAKDAPCQEEIYRADDPTFDLRKLLPAPTNTEEDAGPYFCMGLVLGSDPDDETNTDVTIHRLCVQSRDEMSIFFAPGRHIDAYRQKAEAAGKPLPISVNMGLDPAIHIGACFEAPTTPFGFDELCVAGGLRGKPVELVNCVTVQQKAIARAEIVIEGEVLPNVRVAEDQNTHTGYAMPEFPGYTGPANPSLPVIKVTAVTMRHNAILQTLVGPGEEHVNLAGIPTEASIYNAVELALPGLLQNVYSHSSGGGKFLAILQIKKRVAGDDGSARQAALIALAVYREVKNIILVDEDVDLFDSDDVLWAMQTRYQGDTGTIVVPGITGHVLDPSQIPEYSPSIHTKGSTCKTIFDCTVPFALKEHFKRAQFRELDPRPFAPELFNEP

SEQ ID NO: 16 - protein, 492 aa, Phascolarctobacterium sp.
MTTKINDLRSALDYLRTIPGQLVETNVEADPRAEISGIYRYVGAKGTVKRPTRLGPAMIFNNVKGHPGAKVAIGVLSSRARVGYLLGCEPEKLGFLLKDSVSTPIAPVVVSADQAPCQEVVHLATEEGFDIRKLIPAPTNTEEDAGPYVTMGLCYGTDPETGDTDITIHRLCLQGKDEISMYFVPGRHLDVFRQKYEKAGKPMPISISIGVDPAIEIAACFEPPTTPLGFNELSIAGSIRGEGVQMVQCKTINEKAIARAEYVIEGELLPDVRVREDQNSNTGKAMPEFPGYTGAMKPAIPLIKVKAVTHRRDPIMQSCIGPSEEHVNMAGIPTEASILGMTEKALPGNVKNVYAHCSGGGKYMAVIQFVKKAPPDEGRQRQAALLAFSAFSELKHVILVDDDVDLFDTDDVLWALNTRFQGDVDVITIPGVRCHPLDPSQSPEFSPSIRDVGISCKTIFDCTVPFGLKEHFQRSKFKEVNPAKWVPELFKK

SEQ ID NO: 17 - protein, 497 aa, Escherichia coli K-12
MDAMKYNDLRDFLTLLEQQGELKRITLPVDPHLEITEIADRTLRAGGPALLFENPKGYSMPVLCNLFGTPKRVAMGMGQEDVSALREVGKLLAFLKEPEPPKGFRDLFDKLPQFKQVLNMPTKRLRGAPCQQKIVSGDDVDLNRIPIMTCWPEDAAPLITWGLTVTRGPHKERQNLGIYRQQLIGKNKLIMRWLSHRGGALDYQEWCAAHPGERFPVSVALGADPATILGAVTPVPDTLSEYAFAGLLRGTKTEVVKCISNDLEVPASAEIVLEGYIEQGETAPEGPYGDHTGYYNEVDSFPVFTVTHITQREDAIYHSTYTGRPPDEPAVLGVALNEVFVPILQKQFPEIVDFYLPPEGCSYRLAVVTIKKQYAGHAKRVMMGVWSFLRQFMYTKFVIVCDDDVNARDWNDVIWAITTRMDPARDTVLVENTPIDYLDFASPVSGLGSKMGLDATNKWPGETQREWGRPIKKDPDVVAHIDAIWDELAIFNNGKSA

SEQ ID NO: 18 - protein, 473 aa, Bacillus megaterium QM B1551
MAYKDFRDFLNTLHKEGQLLTVTDEVQPDPDLGSAGQAISNLGDQTPGLLFTNIYGYNNAKVALNVMGSWSNHALMMGLPKSTPVKEQFFEFARRYEKFPVKVKREETAPFHECEIKDDINLFDLLPLFRLNQGDGGYYLDKACVISRDQHDKENFGKQNVGIYRMQVKGKDRLGIQPVPQHDIAIHLKQAEEKGENLPVSIALGCEPAIVTAAATPLHYDQSEYEMAGAIQGEPYRIVKSQLSDLDVPWGAEVILEGEILAGEREYEGPFGEFTGHYSGGRSMPVIKINRVYHRKDPIFESLYIGMPWTETDYLIGINTSVPLYQQLKEAYPEEIEAVNAMYTHGLVAIVSTKSRYGGFAKAVGMRALTTPHGLGYCKLVILVDEDVDPFNLPQVMWALSTKMHPKHDVITVPNLSVLPLDPGSEPAGITDKMILDATTPVAPETRGHYSQPLDTPLETEKWEKILTNMMQK

SEQ ID NO: 19 - protein, 423 aa, Methanothermobacter sp. CaT2
MRNFLDKIGEEALVVEDEVSTSFEAASILREHPRDLVILKNLKESDIPVISGLCNTREKIALSLNCRVHEITHRIVEAMENPTPISSVGGLDGYRSGRADLSELPILRHYRRDGGPYITAGVIFARDPDTGVRNASIHRMMVIGDDRLAVRIVPRHLYTYLQKAEERGEDLEIAIAIGMDPATLLATTTSIPIDADEMEVANTFHEGELELVRCEGVDMEVPPAEIILEGRILCGVREREGPFVDLTDTYDVVRDEPVISLERMHIRKDAMYHAILPAGFEHRLLQGLPQEPRIYRAVKNTVPTVRNVVLTEGGCCWLHAAVSIKKQTEGDGKNVIMAALAAHPSLKHVVVVDEDIDVLDPEEIEYAIATRVKGDDDILIVPGARGSSLDPAALPDGTTTKVGVDATAPLASAEKFQRVSRSE

SEQ ID NO: 20 - protein, 494 aa, Mycobacterium chelonae
  Mycobacterium chelonae 1518
MAFNDLRRYLADLEAHGELRTIKTPVSTEIQLGAIARLACETYGPAALFENLVGYPTFRGLAAFETYSGNPDNRAWRLARALGLSDDTTGDQIVDFLAGFRDTAGVAPVLVETGPVHENIVRDRGELLDYLPIPHLHPGDGGPYVNTIGFFVLESPDRSWVNWAVARCMKLDGDRMVGMTAVMQHIGMLRREWDKIGTSVPFALVLGADPITTLISGGPLAKFGASEGDIIGAIRGEPLEVVECVTSSLRVPAHAEIVIEGYIDLTESADEGPMAEYHGYIDKAKNTTGAPDFGVYHITAVTHRNDAIYPSTCAGKPVDEDHTITGPGVAAASLNALRAASLPVEKAWMVPESASHVLAVTVSDGWSGEFPDANELCRKIGNAVKTMDHSAYWVQRILVTDNDIDPTSPSDLWWAYATRCRPGDDSIILEDVPIMALSPIVNTREERTKTRGRVEVLNCLIPPYADDLSVTSAALRQAYPHDAIAFAERTYLGE

SEQ ID NO: 21 - protein, 512 aa, Hypocrea atroviridis
  Hypocrea atroviridis (strain ATCC 20476)
MSSTTYKSEAFDPEPPHLSFRSFVEALRQDNDLVDINEPVDPDLEAAAITRLVCETDDKAPLFNNVIGAKDGLWRILGAPASLRSSPKERFGRLARHLALPPTASAKDILDKMLSANSIPPIEPVIVPTGPVKENSIEGENIDLEALPAPMVHQSDGGKYIQTYGMHVIQSPDGCWTNWSIARAMVSGKRTLAGLVISPQHIRKIQDQWRAIGQEEIPWALAFGVPPTAIMASSMPIPDGVSEAGYVGAIAGEPIKLVKCDTNNLYVPANSEIVLEGTLSTTKMAPEGPFGEMHGYVYPGESHPGPVYTVNKITYRNNAILPMSACGRLTDETQTMIGTLAAAEIRQLCQDAGLPITDAFAPFVGQATWVALKVDTKRLRAMKTNGKAFAKRVGDVVFTQKPGFTIHRLILVGDDIDVYDDKDVMWAFTTRCRPGTDEVFFDDVVGFQLIPYMSHGNAEAIKGGKVVSDALLTAEYTTGKDWESADFKNSYPKSIQDKVLNSWERLGFKKLD

SEQ ID NO: 22 - protein, 508 aa, Sphaerulina
  Sphaerulina musiva (strain SO2202)
MSSSKQQHLSHANQELPHLNFRSFVQALKDDGDLIEIDDEIDPHLEAGAIIRRACETDGKAPLLNNLKGAKDGLWRILGAPASLRSDPSQKYGRVARHLALPPTATMKDILDKMLSAAHAEPIPPNIVESGPVKENKLVDGEFDLSTLPAPWLHQADGGKYIQTYGMHIVQSPDGKWTNWSIARAMVHDKNHLTGLVIEPQHIWQIHQQWKKVGKDVPWALAFGVPPAAIMAASMPIPDGVTEAGYIGAMTGSALDVVKCETNGMYVPANAEIVLEGTLSITETAPEGPFGEMHGYVFPGDTHPWPKYKVDAITYRNGAILPVSNCGRITDETHTLIGPLAAAQIRQLCQDAGLPITDAFAPFHTQVTWVALKVDIEKLGKMNTTPEAFRKQVGDLVFNHKAGYTIHRLVLCGSDIDVYEWDDIAFAFSTRCRPNKDETFYEDCQGFPLIPYMSHGTGSPIKGGKVISDALMPSEYRGQQDWQQASFKHSYPESLQKSVIERWASWGF

SEQ ID NO: 23 - protein, 498 aa, Penicillium roqueforti
MANIEPHLCFRSFVEALKADNDLVEIDTPIDPNLEAAAITRLVCETNDKAPLFNNIIGTEKGLFRILGAPASLRNSSKDRYGRLARHLALPPTASMRDILDKMLSAGTPIPPNIVSTGPCKENFLEESQIDLTKLPAPLIHQADGGKYIQTYGMHIVQSPDGSWTNWSIARAMVSDDKHLTGLVIEPQHLWQIHQMWKKEGRDAPWALAFGVPPAAIMASSMPIPDGVSEAGYVGSMTGSALDLVKCDTNDLYVPATSEIVFEGTLSITEKGPEGPFGEMHGYVFPGDVHLCPKYKVNRITYRNDPIMPMSSCGRLTDETHTMIGSLAAAVIRKICQQAGLPVNDAFAPFESQVTWVALRIDTAKLREMKTTPKEFSKKVGELIFNSKAGYTIHRLVLCGDDIDVYNGKDVMWAFSTRCRPNLDEIFFEDVPGFPLIPYMSHGNGSPVKGGKVVSDALLPCEYTTGKNWEAADFESSYPEAVKQKVLANWTKMGFREE

SEQ ID NO: 24 - protein, 503 aa, Fusarium oxysporum f. sp. lycopersici
MPSKTLPHMDFRSYVEALEADGDLVSITEECDPHLEVGAIIRKVVENNDKAPLFNKLKGQDENGFWRILGAPNSLRSDPKQRYGRLARHLGLPTDSSMKVILDKMIAAKTTPPIPPTVVETGPCKEHILTPDQFDLTKLPAPLLHQSDGGKYIQTYGMHIVQSPDGKWTNWSIARAMVYDRNHLAGLVIKPQHLYQIHEMWKKEGRDMPWALAFGVPPAAIMASSMPLPDGLSEAEYIGSLVGSSLDVIKCETNGLYVPANSEIVFEGTCSITETAPEGPFGEMHGYVFPGDAHPWPKYTVDLITHRKDAILPVSNCGRLTDETHTMIGPLAAAEIGFLLKSKGLPIKEAFSPFESQVTWVALQVDTQKLREMKTTSEKFCREIGDIIFNHKVGYTIHRLVIVGDDINVYDFKDVIWAFCTRCRPGTDEYFFEDVAGFPLIPYMSHGNGAPNRGGKVVSDSLLPVEYTTGKNWEAADFENSFPEEIKDRVCSRWQTLGFSSAK

SEQ ID NO: 25 - protein, 503 aa, Saccharomyces kudriavzevii
  Saccharomyces kudriavzevii (strain ATCC MYA-4449)
MSALNPALQFRDFIQVLKDEDDLIEITKEVDPNLEVGAIMRKAYESKLPAPFFKNIKGASKDLFNILGCPAGLRNKKKGDHGRIAHHLGLDPKTTIKEIIDYLLECKNKKPLPPSSISASSAPCKAHVLSEEEIHLESLPTPYLHTSDGGNYLQTYGMWILQTPDKKWTNWSIARGMVVDDKHITGLVIKPQHIRQIADAWGAIGKGNKIPFALCFGVPPAAILVSSMPIPEGVSESDYVGAILGKPVPVVKCETNDLMVPATSEIVFEGTLSLTDTHAEGPFGEMHGYVFGGQGHPCPLYTVKAMTHRDNAILPVSNPGLCTDETHTLIGSLVATEAKELAIKSGLPVLDAFTPYEAQALWLVLKVDLKRLQALKTTPEEFSKKVGDIYFRTKVGFIIHEIVLVADDIDIFNFKEVFWAYVTRHTPVADQTAFDDVTSFPLAPFVSQSPRSKTMKGGKCVTNCIFRQQYERDFDYVTCSFEKGYSKELVDRINENWREYGYK

SEQ ID NO: 26 - protein, 503 aa, Saccharomyces cerevisiae S288c; identical to SEQ ID NO: 9

SEQ ID NO: 27 - protein, 503 aa, Aspergillus parasiticus
MAAISEVDHSFRAFVEALKADDDLVEINTEIDSNLEAAAITRLVCETDDKAPLFNNLKGMGKNGLFRILGAPGSLRKSKRDRYGRLARHLALPPTASMKEILDKMLSASQLPPIDPKIVETGPVKENSLEGDEIDLTALPVPMVHKSDGGKYLQTYGMHIVQSPDGKWTNWSIARAMVKDKNHLTGLVIEPQHIWQIHQMWKKEGKDVPWALCFGVPPAAIMASSMPIPDGVTEAGYVGAMTGRALELVKCDTNHLYVPANAEIVLEGTLSITETADEGPFGEMHGYVFPGDSHKCPVYKVNKITYRTDAILPMSACGRLTDETHTMIGSLAAAEIRKICQLAGLPITDTFSPFEAQVTWVALKVDTAKLRQMNLTPKELQKWVGDVVFNHKAGYTIHRLVLVGDDIDPYEWKDVMWAFATRCRPNADEMFFEDVRGFPLIPYMGHGTGSPTKGGKVVSDALMPTEYTTGADWEAADFEHSYPEEIKAKVRAQWQALGFRKQE

SEQ ID NO: 28 - protein, 513 aa, Candida albicans
MSLNPALKFRDFIQVLKNEGDLVEIDTEVDPNLEVGAITRKAYENKLAAPLFNNLKQDPGNVDPKNLFRILGCPGGLRGFGNDHARIALHLGLDSQTPMKEIVDFLVANRNPKKFIPPVLVPNEKSPHKKHHLTHEQIDLTKLPVPLLHHGDGGKFIQTYGMWVLQTPDKSWTNWSIARGMVHDSKSITGLVINPQHVKQVSDAWVAAGKGDKIPFALCFGVPPAAILVSSMPIPDGATEAEYIGGLCNQAVPVVKCETNDLEVPADCEMVFEGYLDRDTLVTEGPFGEMHGYCFPQDHHTQPLYRVNHISYRDEAIMPISNPGLCTDETHTLIGGLVSAETKYLISQHLVLSKIVEDVFTPYEAQALWLAVKINIQELIKLKTNAKELSNLVGDFLFKSKECYKVCSILHEVILVGDDIDIFDFKQLIWAYTTRHTPVQDQVYFDDVKPFPLAPFISQGSLIKTRQGGKCVTSCIFPKQFTDPDFKFVTCNFDGYPEEVKNKVSQNWEKYYK

SEQ ID NO: 29 - protein, 500 aa, Grosmannia clavigera kw1407
MASSQDLPHMSFRAFVDELRADGDIVEINDECDADLEVGAIIRLACETDAKAPLFNKLKGMDGNGLWRILGAPNSLRADPAQRFGRLARHINLPPTASMKEILDKMGAAKSTPPIPPKTVPTGSCKEVKLTPDQFDLTTLPSPQLHKSDGGKYVQTYGMHIVQTPDGKWTNWSIARAMVHDRNHLVGLVIPPQHIWKVQQEWKKIGKDMPWALVFGVPPAAIMAASMPLPDGLSEAEYIGSLVGTALEVTKCDTNDLLVPANSEIVFEGFMSSTETAPEGPFGEMHGYVFPGDAHPQPLYTVNMITHRKDAILPVSNCGRLTDETHTMIGPLVAVEINVMLKAAGLPITDAYTPFESQVTWCAVKVDTAKLRELKTTPKEFCRKIGDLIFNTKVGSTIHRIAVVGDDIDIFNFKDVIWAFCTRCRPGMDEYLFEDVPGFPLIPYMSHGNGPANRGGKVVSDCLLPKEYTTGKNWEAASFKESIPESVQAKVLGNWKAWGF

SEQ ID NO: 30 - protein, 496 aa, Enterobacter cloacae
MENQINDLRSAIALLQRHEGQYIETDRPVDPNAELAGVYRHIGAGGTVKRPTRTGPAMMFNSIKGYPHSRILVGMHASRERAALLLGCEPSELAKHVGQAVKKPVAPVVVPASQAPCQEQVFYADDPDFDLRKLLPAPTNTPIDAGPFFCLGLVLASDPEDSSLTDVTIHRLCVQERDELSMFLAAGRHIEVFRKKAEDAGKPLPVTINMGLDPAIYIGACFEAPTTPFGYNELGVAGALRQQPVELVQGVAVKEKAIARAEIIIEGELLPGVRVREDQHTNTGHAMPEFPGYCGEANPSLPVIKVKAVTMRNHAILQTLVGPGEEHTTLAGLPTEASIRNAVEEAIPGFLQNVYAHTAGGGKFLGILQVKKRQPSDEGRQGQAALIALATYSELKNIILVDEDVDIFDSDDILWAMTTRMQGDVSITNIPGIRGHQLDPSQSPDYSTSIRGNGISCKTIFDCTVPWALKDRFERAPFMEVDPRPWAPELFADNTK

SEQ ID NO: 31 - protein, 262 aa, Escherichia coli (strain K12)
MQVDLLGSAQSAHALHLFHQHSPLVHCMTNDVVQTFTANTLLALGASPAMVIETEEASQFAAIASALLINVGTLTQPRAQAMRAAVEQAKSSQTPWTLDPVAVGALDYRRHFCHELLSFKPAAIRGNASEIMALAGIANGGRGVDTTDAAANAIPAAQTLARETGAIVVVTGEMDYVTDGHRIIGIHGGDPLMTKVVGTGCALSAVVAACCALPGDTLENVASACHWMKQAGERAVARSEGPGSFVPHFLDALWQLTQEVQA

SEQ ID NO: 32 - protein, 272 aa, Bacillus subtilis
MDAQSAAKCLTAVRRHSPLVHSITNNVVTNFTANGLLALGASPVMAYAKEEVADMAKIAGALVLNIGTLSKESVEAMIIAGKSANEHGVPVILDPVGAGATPFRTESARDIIREVRLAAIRGNAAEIAHTVGVTDWLIKGVDAGEGGGDIIRLAQQAAQKLNTVIAITGEVDVIADTSHVYTLHNGHKLLTKVTGAGCLLTSVVGAFCAVEENPLFAAIAAISSYGVAAQLAAQQTADKGPGSFQIELLNKLSTVTEQDVQEWATIERVTVS

SEQ ID NO: 33 - protein, 267 aa, Rhizobium leguminosarum bv. viciae (strain 3841)
MQTRTTPGAMLKAMREKPPLVQCITNYVAMNIAANVLLAAGASPAMVHAAEEAGEFAAIASALTINIGTLSTQWIDGMQAAAKAATSAGKPWVLDPVAHYATAFRRNAVAELLALKPTIIRGNASEIIALAGGESRGQGVDSRDPVEQAEGSARWLAERQRAVVAVTGAVDFVTDGERAVRIEGGSALMPQVTALGCSLTCLVGAFAATAPEDIFGATVAALSTFAIAGEEAALGAAGPGSFSWRFLDALAALDAETLDARARISAA

SEQ ID NO: 34 - protein, 313 aa, Escherichia coli (strain K12)
MKLIRGIHNLSQAPQEGCVLTIGNFDGVHRGHRALLQGLQEEGRKRNLPVMVMLFEPQPLELFATDKAPARLTRLREKLRYLAECGVDYVLCVRFDRRFAALTAQNFISDLLVKHLRVKFLAVGDDFRFGAGREGDFLLLQKAGMEYGFDITSTQTFCEGGVRISSTAVRQALADDNLALAESLLGHPFAISGRVVHGDELGRTIGFPTANVPLRRQVSPVKGVYAVEVLGLGEKPLPGVANIGTRPTVAGIRQQLEVHLLDVAMDLYGRHIQVVLRKKIRNEQRFASLDELKAQIARDELTAREFFGLTKPA

SEQ ID NO: 35 - protein, 512 aa, Hypocrea atroviridis
MSSTTYKSEAFDPEPPHLSFRSFVNALRQDGDLVDINEPVDPDLEAAAITRLVCETDDKAPLFNNVIGAKDGLWRILGAPASLRASPKERFGRLARHLALPPTASAKDILDKMLSANSIPPIEPVIVPTGPVKENSIEGENIDLEALPAPMVHQSDGGKYINTYGMHVIQSPDGGWTNWSIARAMVSGKRTLAGLVISPQHIRKIQDQWRAIGQEEIPWALAFGVPPLAIMASSMPIPDGVSEAGYVGAIAGEPIKLVKCDTNNLYVPANSEIVLEGTLSTTKMAPEGPFGEMHGYVYPGESHPGPVYTVNKITYRNNAILPMSACGRLTDETQTMIPTLAAAEIRQLCQRAGLPITDAFAPFVGQATWVALKVDTKRLRAMKTNGKAFAKAVGDVVFTQKPGFMIHRLILVGDDIDVYDDKDVMWAFATRCRPGTDEVFFDDVPGFWLIPYMSHGNAEAVKGGKVVSDALLTAEYTTGKDWESADFKNSYPKRIQDKVLNSWERLGFKKLD

SEQ ID NO: 36 - DNA, 7452 bp, Artificial Sequence
  pGB6346
ctctcccttatgcgactcctgcattaggaagcagcccagtagtaggttgaggccgttgagcaccgccgccgcaaggaatggtgcatgcaaggagatggcgcccaacagtcccccggccacggggcctgccaccatacccacgccgaaacaagcgctcatgagcccgaagtggcgagcccgatcttccccatcggtgatgtcggcgatataggcgccagcaaccgcacctgtggcgccggtgatgccggccacgatgcgtccggcgtagaggatcgagatcgatctcgatcccgcgaaattaatacgactcactataggggaattgtgagcggataacaattcccctctagaaataattttgtttaactttaagaaggagatataccatgagcagcaccacctataaaagtgaagcatttgatccggaaccgcctcatctgagctttcgtagctttgttaatgcactgcgtcaggatggggatctggtggatattaatgaaccggttgatccggatctggaagcagcagcaattacccgtctggtttgtgaaaccgatgataaagcaccgctgtttaataacgtgattggtgcaaaagatggtctgtggcgtattctgggtgcaccggcaagcctgcgtgcgagcccgaaagaacgttttggtcgtctggcacgtcatctggcactgcctccgaccgcaagcgcaaaagatattctggataaaatgctgagcgccaatagcattccgcctattgaaccggttattgttccgaccggtccggttaaagaaaatagcattgaaggcgaaaacattgatctggaagccctgcctgcaccgatggttcatcagagtgatggtggcaagtatatcaatacctatggtatgcatgttatccagagtccggatggtgggtggaccaattggagcattgcccgtgcaatggttagcggtaaacgtaccctggcaggtctggttattagtccgcagcatattcgtaaaattcaggatcagtggcgtgcaattggccaagaagaaattccttgggcactggcatttggtgttccgcctctggcaattatggcaagcagtatgccgattccggatggtgttagcgaagcaggttatgttggtgcaattgccggtgaaccgattaaactggttaaatgcgataccaacaatctgtatgttccggcaaatagcgaaattgttctggaaggcaccctgagcaccaccaaaatggcaccggaaggtccgtttggtgaaatgcatggttatgtttatccgggtgaaagccatccgggtccggtttataccgttaacaaaattacctatcgcaacaatgcaattctgccgatgagcgcatgtggtcgtctgaccgatgaaacccagaccatgattccgaccctggcagcagcagaaattcgtcagctgtgtcagagggcaggtctgccgattaccgatgcatttgcaccgtttgttggtcaggcaacctgggttgcactgaaagttgataccaaacgtctgcgtgcaatgaaaaccaatggtaaagcatttgcaaaagcggttggtgatgttgtgtttacccagaaaccgggttttatgattcatcgtctgattctggttggtgatgatattgatgtgtatgacgataaagatgtgatgtgggcatttgctacccgttgtcgtccgggtacagatgaagttttttttgatgatgttcctggcttttggctgatcccgtatatgagtcatggtaatgccgaagcagtgaaaggtggtaaagttgttagtgatgcactgctgaccgcagaatataccaccggtaaagattgggaaagcgcagatttcaaaaacagctatccgaaacgtatccaggataaagttctgaatagctgggaacgcctgggtttcaaaaaactggattaataaggatccgaattcgagctcggcgcgcctgcaggtcgacaagcttgcggccgcataatgcttaagtcgaacagaaagtaatcgtattgtacacggccgcataatcgaaattaatacgactcactataggggaattgtgagcggataacaattccccatcttagtatattagttaagtataagaaggagatatacatatgaaacgactcattgtaggcatcagcggtgccagcggcgcgatttatggcgtgcgcttattacaggttctgcgcgatgtcacagatatcgaaacgcatctggtgatgagccaggcagcgcgccagaccttatccctcgaaacggatttttctctgcgcgaagtgcaggcattagccgatgtcacgcacgatgcgcgcgatattgccgccagcatctcttccggttctttccagacgctggggatggtgattttaccctgttcaatcaaaaccctttccggcattgtccatagctatactgatggcttactgacccgtgcggcagatgtggtgctgaaagagcgtcgcccgttggtgctctgcgtgcgtgaaacaccattgcacttaggccatctgcgtttaatgactcaggcggcagaaatcggtgcggtgattatgcctcccgttccggcgttttatcatcgcccgcaatcccttgatgatgtgataaatcagacggttaatcgtgttcttgaccagtttgcgataacccttcctgaagatctctttgcccgctggcagggcgcataataaggtaccctcgagtctggtaaagaaaccgctgctgcgaaatttgaacgccagcacatggactcgtctactagcgcagcttaattaacctaggctgctgccaccgctgagcaataactagcataaccccttggggcctctaaacgggtcttgaggggttttttgctgaaaggaggaactatatccggattggcgaatgggacgcgccctgtagcggcgcattaagcgcggcgggtgtggtggttacgcgcagcgtgaccgctacacttgccagcgccctagcgcccgctcctttcgctttcttcccttcctttctcgccacgttcgccggctttccccgtcaagctctaaatcgggggctccctttagggttccgatttagtgctttacggcacctcgaccccaaaaaacttgattagggtgatggttcacgtagtgggccatcgccctgatagacggtttttcgccctttgacgttggagtccacgttctttaatagtggactcttgttccaaactggaacaacactcaaccctatctcggtctattcttttgatttataagggattttgccgatttcggcctattggttaaaaaatgagctgatttaacaaaaatttaacgcgaattttaacaaaatattaacgtttacaatttctggcggcacgatggcatgagattatcaaaaaggatcttcacctagatccttttaaattaaaaatgaagttttaaatcaatctaaagtatatatgagtaaacttggtctgacagttaccaatgcttaatcagtgaggcacctatctcagcgatctgtctatttcgttcatccatagttgcctgactccccgtcgtgtagataactacgatacgggagggcttaccatctggccccagtgctgcaatgataccgcgagacccacgctcaccggctccagatttatcagcaataaaccagccagccggaagggccgagcgcagaagtggtcctgcaactttatccgcctccatccagtctattaattgttgccgggaagctagagtaagtagttcgccagttaatagtttgcgcaacgttgttgccattgctacaggcatcgtggtgtcacgctcgtcgtttggtatggcttcattcagctccggttcccaacgatcaaggcgagttacatgatcccccatgttgtgcaaaaaagcggttagctccttcggtcctccgatcgttgtcagaagtaagttggccgcagtgttatcactcatggttatggcagcactgcataattctcttactgtcatgccatccgtaagatgcttttctgtgactggtgagtactcaaccaagtcattctgagaatagtgtatgcggcgaccgagttgctcttgcccggcgtcaatacgggataataccgcgccacatagcagaactttaaaagtgctcatcattggaaaacgttcttcggggcgaaaactctcaaggatcttaccgctgttgagatccagttcgatgtaacccactcgtgcacccaactgatcttcagcatcttttactttcaccagcgtttctgggtgagcaaaaacaggaaggcaaaatgccgcaaaaaagggaataagggcgacacggaaatgttgaatactcatactcttcctttttcaatcatgattgaagcatttatcagggttattgtctcatgagcggatacatatttgaatgtatttagaaaaataaacaaataggtcatgaccaaaatcccttaacgtgagttttcgttccactgagcgtcagaccccgtagaaaagatcaaaggatcttcttgagatcctttttttctgcgcgtaatctgctgcttgcaaacaaaaaaaccaccgctaccagcggtggtttgtttgccggatcaagagctaccaactctttttccgaaggtaactggcttcagcagagcgcagataccaaatactgtccttctagtgtagccgtagttaggccaccacttcaagaactctgtagcaccgcctacatacctcgctctgctaatcctgttaccagtggctgctgccagtggcgataagtcgtgtcttaccgggttggactcaagacgatagttaccggataaggcgcagcggtcgggctgaacggggggttcgtgcacacagcccagcttggagcgaacgacctacaccgaactgagatacctacagcgtgagctatgagaaagcgccacgcttcccgaagggagaaaggcggacaggtatccggtaagcggcagggtcggaacaggagagcgcacgagggagcttccagggggaaacgcctggtatctttatagtcctgtcgggtttcgccacctctgacttgagcgtcgatttttgtgatgctcgtcaggggggcggagcctatggaaaaacgccagcaacgcggcctttttacggttcctggccttttgctggccttttgctcacatgttctttcctgcgttatcccctgattctgtggataaccgtattaccgcctttgagtgagctgataccgctcgccgcagccgaacgaccgagcgcagcgagtcagtgagcgaggaagcggaagagcgcctgatgcggtattttctccttacgcatctgtgcggtatttcacaccgcatatatggtgcactctcagtacaatctgctctgatgccgcatagttaagccagtatacactccgctatcgctacgtgactgggtcatggctgcgccccgacacccgccaacacccgctgacgcgccctgacgggcttgtctgctcccggcatccgcttacagacaagctgtgaccgtctccgggagctgcatgtgtcagaggttttcaccgtcatcaccgaaacgcgcgaggcagctgcggtaaagctcatcagcgtggtcgtgaagcgattcacagatgtctgcctgttcatccgcgtccagctcgttgagtttctccagaagcgttaatgtctggcttctgataaagcgggccatgttaagggcggttttttcctgtttggtcactgatgcctccgtgtaagggggatttctgttcatgggggtaatgataccgatgaaacgagagaggatgctcacgatacgggttactgatgatgaacatgcccggttactggaacgttgtgagggtaaacaactggcggtatggatgcggcgggaccagagaaaaatcactcagggtcaatgccagcgcttcgttaatacagatgtaggtgttccacagggtagccagcagcatcctgcgatgcagatccggaacataatggtgcagggcgctgacttccgcgtttccagactttacgaaacacggaaaccgaagaccattcatgttgttgctcaggtcgcagacgttttgcagcagcagtcgcttcacgttcgctcgcgtatcggtgattcattctgctaaccagtaaggcaaccccgccagcctagccgggtcctcaacgacaggagcacgatcatgctagtcatgccccgcgcccaccggaaggagctgactgggttgaaggctctcaagggcatcggtcgagatcccggtgcctaatgagtgagctaacttacattaattgcgttgcgctcactgcccgctttccagtcgggaaacctgtcgtgccagctgcattaatgaatcggccaacgcgcggggagaggcggtttgcgtattgggcgccagggtggtttttcttttcaccagtgagacgggcaacagctgattgcccttcaccgcctggccctgagagagttgcagcaagcggtccacgctggtttgccccagcaggcgaaaatcctgtttgatggtggttaacggcgggatataacatgagctgtcttcggtatcgtcgtatcccactaccgagatgtccgcaccaacgcgcagcccggactcggtaatggcgcgcattgcgcccagcgccatctgatcgttggcaaccagcatcgcagtgggaacgatgccctcattcagcatttgcatggtttgttgaaaaccggacatggcactccagtcgccttcccgttccgctatcggctgaatttgattgcgagtgagatatttatgccagccagccagacgcagacgcgccgagacagaacttaatgggcccgctaacagcgcgatttgctggtgacccaatgcgaccagatgctccacgcccagtcgcgtaccgtcttcatgggagaaaataatactgttgatgggtgtctggtcagagacatcaagaaataacgccggaacattagtgcaggcagcttccacagcaatggcatcctggtcatccagcggatagttaatgatcagcccactgacgcgttgcgcgagaagattgtgcaccgccgctttacaggcttcgacgccgcttcgttctaccatcgacaccaccacgctggcacccagttgatcggcgcgagatttaatcgccgcgacaatttgcgacggcgcgtgcagggccagactggaggtggcaacgccaatcagcaacgactgtttgcccgccagttgttgtgccacgcggttgggaatgtaattcagctccgccatcgccgcttccactttttcccgcgttttcgcagaaacgtggctggcctggttcaccacgcgggaaacggtctgataagagacaccggcatactctgcgacatcgtataacgttactggtttcacattcaccaccctgaattgactctcttccgggcgctatcatgccataccgcgaaaggttttgcgccattcgatggtgtccgggatctcgacg

SEQ ID NO: 37 - DNA, 8182 bp, Artificial Sequence
  pGB6580
caccgccgccgcaaggaatggtgcatgcaaggagatggcgcccaacagtcccccggccacggggcctgccaccatacccacgccgaaacaagcgctcatgagcccgaagtggcgagcccgatcttccccatcggtgatgtcggcgatataggcgccagcaaccgcacctgtggcgccggtgatgccggccacgatgcgtccggcgtagaggatcgagatcgatctcgatcccgcgaaattaatacgactcactataggggaattgtgagcggataacaattcccctctagaaataattttgtttaactttaagaaggagatataccatgagcagcaccacctataaaagtgaagcatttgatccggaaccgcctcatctgagctttcgtagctttgttaatgcactgcgtcaggatggggatctggtggatattaatgaaccggttgatccggatctggaagcagcagcaattacccgtctggtttgtgaaaccgatgataaagcaccgctgtttaataacgtgattggtgcaaaagatggtctgtggcgtattctgggtgcaccggcaagcctgcgtgcgagcccgaaagaacgttttggtcgtctggcacgtcatctggcactgcctccgaccgcaagcgcaaaagatattctggataaaatgctgagcgccaatagcattccgcctattgaaccggttattgttccgaccggtccggttaaagaaaatagcattgaaggcgaaaacattgatctggaagccctgcctgcaccgatggttcatcagagtgatggtggcaagtatatcaatacctatggtatgcatgttatccagagtccggatggtgggtggaccaattggagcattgcccgtgcaatggttagcggtaaacgtaccctggcaggtctggttattagtccgcagcatattcgtaaaattcaggatcagtggcgtgcaattggccaagaagaaattccttgggcactggcatttggtgttccgcctctggcaattatggcaagcagtatgccgattccggatggtgttagcgaagcaggttatgttggtgcaattgccggtgaaccgattaaactggttaaatgcgataccaacaatctgtatgttccggcaaatagcgaaattgttctggaaggcaccctgagcaccaccaaaatggcaccggaaggtccgtttggtgaaatgcatggttatgtttatccgggtgaaagccatccgggtccggtttataccgttaacaaaattacctatcgcaacaatgcaattctgccgatgagcgcatgtggtcgtctgaccgatgaaacccagaccatgattccgaccctggcagcagcagaaattcgtcagctgtgtcagagggcaggtctgccgattaccgatgcatttgcaccgtttgttggtcaggcaacctgggttgcactgaaagttgataccaaacgtctgcgtgcaatgaaaaccaatggtaaagcatttgcaaaagcggttggtgatgttgtgtttacccagaaaccgggttttatgattcatcgtctgattctggttggtgatgatattgatgtgtatgacgataaagatgtgatgtgggcatttgctacccgttgtcgtccgggtacagatgaagttttttttgatgatgttcctggcttttggctgatcccgtatatgagtcatggtaatgccgaagcagtgaaaggtggtaaagttgttagtgatgcactgctgaccgcagaatataccaccggtaaagattgggaaagcgcagatttcaaaaacagctatccgaaacgtatccaggataaagttctgaatagctgggaacgcctgggtttcaaaaaactggattaataaggatccgaattcgagctcggcgcgcctgcaggtcgacaagcttgcggccgcataatgcttaagtcgaacagaaagtaatcgtattgtacacggccgcataatcgaaattaatacgactcactataggggaattgtgagcggataacaattccccatcttagtatattagttaagtataagaaggagatatacatatgaaacgactcattgtaggcatcagcggtgccagcggcgcgatttatggcgtgcgcttattacaggttctgcgcgatgtcacagatatcgaaacgcatctggtgatgagccaggcagcgcgccagaccttatccctcgaaacggatttttctctgcgcgaagtgcaggcattagccgatgtcacgcacgatgcgcgcgatattgccgccagcatctcttccggttctttccagacgctggggatggtgattttaccctgttcaatcaaaaccctttccggcattgtccatagctatactgatggcttactgacccgtgcggcagatgtggtgctgaaagagcgtcgcccgttggtgctctgcgtgcgtgaaacaccattgcacttaggccatctgcgtttaatgactcaggcggcagaaatcggtgcggtgattatgcctcccgttccggcgttttatcatcgcccgcaatcccttgatgatgtgataaatcagacggttaatcgtgttcttgaccagtttgcgataacccttcctgaagatctctttgcccgctggcagggcgcataataaggtaccgaaggagatatacatatgctgaccattctgaaactgggtggtagcattctgagcgataaaaatgttccgtatagcattaaatgggacaacctggaacgtatcgcaatggaaatcaaaaatgccctggactactacaaaaatcagaataaagaaattaaactgattctggtgcatggtggtggtgcatttggtcatccggttgccaaaaaatacctgaaaattgaggacggcaaaaaaatctttattaacatggaaaaaggcttttgggaaatccagcgtgcaatgcgtcgttttaacaacattatcattgataccctgcagagctatgatattccggcagttagcattcagccgagcagctttgttgtttttggtgataaactgatctttgacaccagcgccattaaagaaatgctgaaacgtaatctggttccggtgattcatggtgatattgtgattgatgataaaaatggctaccgcatcattagcggtgatgatattgttccgtatctggccaatgaactgaaagcagatctgattctgtatgccaccgatgttgatggtgttctgattgataacaaaccgattaaacgcattgataaaaacaatatctataaaatcctgaattatctgagcggcagcaacagcattgatgttaccggtggtatgaaatacaaaatcgacatgattcgcaaaaacaaatgccgtggctttgtgttcaatggcaataaagccaacaacatctataaagcactgctgggtgaagttgaaggcaccgaaattgattttagcgaataataattaattaacctaggctgctgccaccgctgagcaataactagcataaccccttggggcctctaaacgggtcttgaggggttttttgctgaaaggaggaactatatccggattggcgaatgggacgcgccctgtagcggcgcattaagcgcggcgggtgtggtggttacgcgcagcgtgaccgctacacttgccagcgccctagcgcccgctcctttcgctttcttcccttcctttctcgccacgttcgccggctttccccgtcaagctctaaatcgggggctccctttagggttccgatttagtgctttacggcacctcgaccccaaaaaacttgattagggtgatggttcacgtagtgggccatcgccctgatagacggtttttcgccctttgacgttggagtccacgttctttaatagtggactcttgttccaaactggaacaacactcaaccctatctcggtctattcttttgatttataagggattttgccgatttcggcctattggttaaaaaatgagctgatttaacaaaaatttaacgcgaattttaacaaaatattaacgtttacaatttctggcggcacgatggcatgagattatcaaaaaggatcttcacctagatccttttaaattaaaaatgaagttttaaatcaatctaaagtatatatgagtaaacttggtctgacagttaccaatgcttaatcagtgaggcacctatctcagcgatctgtctatttcgttcatccatagttgcctgactccccgtcgtgtagataactacgatacgggagggcttaccatctggccccagtgctgcaatgataccgcgagacccacgctcaccggctccagatttatcagcaataaaccagccagccggaagggccgagcgcagaagtggtcctgcaactttatccgcctccatccagtctattaattgttgccgggaagctagagtaagtagttcgccagttaatagtttgcgcaacgttgttgccattgctacaggcatcgtggtgtcacgctcgtcgtttggtatggcttcattcagctccggttcccaacgatcaaggcgagttacatgatcccccatgttgtgcaaaaaagcggttagctccttcggtcctccgatcgttgtcagaagtaagttggccgcagtgttatcactcatggttatggcagcactgcataattctcttactgtcatgccatccgtaagatgcttttctgtgactggtgagtactcaaccaagtcattctgagaatagtgtatgcggcgaccgagttgctcttgcccggcgtcaatacgggataataccgcgccacatagcagaactttaaaagtgctcatcattggaaaacgttcttcggggcgaaaactctcaaggatcttaccgctgttgagatccagttcgatgtaacccactcgtgcacccaactgatcttcagcatcttttactttcaccagcgtttctgggtgagcaaaaacaggaaggcaaaatgccgcaaaaaagggaataagggcgacacggaaatgttgaatactcatactcttcctttttcaatcatgattgaagcatttatcagggttattgtctcatgagcggatacatatttgaatgtatttagaaaaataaacaaataggtcatgaccaaaatcccttaacgtgagttttcgttccactgagcgtcagaccccgtagaaaagatcaaaggatcttcttgagatcctttttttctgcgcgtaatctgctgcttgcaaacaaaaaaaccaccgctaccagcggtggtttgtttgccggatcaagagctaccaactctttttccgaaggtaactggcttcagcagagcgcagataccaaatactgtccttctagtgtagccgtagttaggccaccacttcaagaactctgtagcaccgcctacatacctcgctctgctaatcctgttaccagtggctgctgccagtggcgataagtcgtgtcttaccgggttggactcaagacgatagttaccggataaggcgcagcggtcgggctgaacggggggttcgtgcacacagcccagcttggagcgaacgacctacaccgaactgagatacctacagcgtgagctatgagaaagcgccacgcttcccgaagggagaaaggcggacaggtatccggtaagcggcagggtcggaacaggagagcgcacgagggagcttccagggggaaacgcctggtatctttatagtcctgtcgggtttcgccacctctgacttgagcgtcgatttttgtgatgctcgtcaggggggcggagcctatggaaaaacgccagcaacgcggcctttttacggttcctggccttttgctggccttttgctcacatgttctttcctgcgttatcccctgattctgtggataaccgtattaccgcctttgagtgagctgataccgctcgccgcagccgaacgaccgagcgcagcgagtcagtgagcgaggaagcggaagagcgcctgatgcggtattttctccttacgcatctgtgcggtatttcacaccgcatatatggtgcactctcagtacaatctgctctgatgccgcatagttaagccagtatacactccgctatcgctacgtgactgggtcatggctgcgccccgacacccgccaacacccgctgacgcgccctgacgggcttgtctgctcccggcatccgcttacagacaagctgtgaccgtctccgggagctgcatgtgtcagaggttttcaccgtcatcaccgaaacgcgcgaggcagctgcggtaaagctcatcagcgtggtcgtgaagcgattcacagatgtctgcctgttcatccgcgtccagctcgttgagtttctccagaagcgttaatgtctggcttctgataaagcgggccatgttaagggcggttttttcctgtttggtcactgatgcctccgtgtaagggggatttctgttcatgggggtaatgataccgatgaaacgagagaggatgctcacgatacgggttactgatgatgaacatgcccggttactggaacgttgtgagggtaaacaactggcggtatggatgcggcgggaccagagaaaaatcactcagggtcaatgccagcgcttcgttaatacagatgtaggtgttccacagggtagccagcagcatcctgcgatgcagatccggaacataatggtgcagggcgctgacttccgcgtttccagactttacgaaacacggaaaccgaagaccattcatgttgttgctcaggtcgcagacgttttgcagcagcagtcgcttcacgttcgctcgcgtatcggtgattcattctgctaaccagtaaggcaaccccgccagcctagccgggtcctcaacgacaggagcacgatcatgctagtcatgccccgcgcccaccggaaggagctgactgggttgaaggctctcaagggcatcggtcgagatcccggtgcctaatgagtgagctaacttacattaattgcgttgcgctcactgcccgctttccagtcgggaaacctgtcgtgccagctgcattaatgaatcggccaacgcgcggggagaggcggtttgcgtattgggcgccagggtggtttttcttttcaccagtgagacgggcaacagctgattgcccttcaccgcctggccctgagagagttgcagcaagcggtccacgctggtttgccccagcaggcgaaaatcctgtttgatggtggttaacggcgggatataacatgagctgtcttcggtatcgtcgtatcccactaccgagatgtccgcaccaacgcgcagcccggactcggtaatggcgcgcattgcgcccagcgccatctgatcgttggcaaccagcatcgcagtgggaacgatgccctcattcagcatttgcatggtttgttgaaaaccggacatggcactccagtcgccttcccgttccgctatcggctgaatttgattgcgagtgagatatttatgccagccagccagacgcagacgcgccgagacagaacttaatgggcccgctaacagcgcgatttgctggtgacccaatgcgaccagatgctccacgcccagtcgcgtaccgtcttcatgggagaaaataatactgttgatgggtgtctggtcagagacatcaagaaataacgccggaacattagtgcaggcagcttccacagcaatggcatcctggtcatccagcggatagttaatgatcagcccactgacgcgttgcgcgagaagattgtgcaccgccgctttacaggcttcgacgccgcttcgttctaccatcgacaccaccacgctggcacccagttgatcggcgcgagatttaatcgccgcgacaatttgcgacggcgcgtgcagggccagactggaggtggcaacgccaatcagcaacgactgtttgcccgccagttgttgtgccacgcggttgggaatgtaattcagctccgccatcgccgcttccactttttcccgcgttttcgcagaaacgtggctggcctggttcaccacgcgggaaacggtctgataagagacaccggcatactctgcgacatcgtataacgttactggtttcacattcaccaccctgaattgactctcttccgggcgctatcatgccataccgcgaaaggttttgcgccattcgatggtgtccgggatctcgacgctctcccttatgcgactcctgcattaggaagcagcccagtagtaggttgaggccgttgag

SEQ ID NO: 38 - DNA, 8188 bp, Artificial Sequence
  pGB6389
caccgccgccgcaaggaatggtgcatgcaaggagatggcgcccaacagtcccccggccacggggcctgccaccatacccacgccgaaacaagcgctcatgagcccgaagtggcgagcccgatcttccccatcggtgatgtcggcgatataggcgccagcaaccgcacctgtggcgccggtgatgccggccacgatgcgtccggcgtagaggatcgagatcgatctcgatcccgcgaaattaatacgactcactataggggaattgtgagcggataacaattcccctctagaaataattttgtttaactttaagaaggagatataccatgagcagcaccacctataaaagtgaagcatttgatccggaaccgcctcatctgagctttcgtagctttgttaatgcactgcgtcaggatggggatctggtggatattaatgaaccggttgatccggatctggaagcagcagcaattacccgtctggtttgtgaaaccgatgataaagcaccgctgtttaataacgtgattggtgcaaaagatggtctgtggcgtattctgggtgcaccggcaagcctgcgtgcgagcccgaaagaacgttttggtcgtctggcacgtcatctggcactgcctccgaccgcaagcgcaaaagatattctggataaaatgctgagcgccaatagcattccgcctattgaaccggttattgttccgaccggtccggttaaagaaaatagcattgaaggcgaaaacattgatctggaagccctgcctgcaccgatggttcatcagagtgatggtggcaagtatatcaatacctatggtatgcatgttatccagagtccggatggtgggtggaccaattggagcattgcccgtgcaatggttagcggtaaacgtaccctggcaggtctggttattagtccgcagcatattcgtaaaattcaggatcagtggcgtgcaattggccaagaagaaattccttgggcactggcatttggtgttccgcctctggcaattatggcaagcagtatgccgattccggatggtgttagcgaagcaggttatgttggtgcaattgccggtgaaccgattaaactggttaaatgcgataccaacaatctgtatgttccggcaaatagcgaaattgttctggaaggcaccctgagcaccaccaaaatggcaccggaaggtccgtttggtgaaatgcatggttatgtttatccgggtgaaagccatccgggtccggtttataccgttaacaaaattacctatcgcaacaatgcaattctgccgatgagcgcatgtggtcgtctgaccgatgaaacccagaccatgattccgaccctggcagcagcagaaattcgtcagctgtgtcagagggcaggtctgccgattaccgatgcatttgcaccgtttgttggtcaggcaacctgggttgcactgaaagttgataccaaacgtctgcgtgcaatgaaaaccaatggtaaagcatttgcaaaagcggttggtgatgttgtgtttacccagaaaccgggttttatgattcatcgtctgattctggttggtgatgatattgatgtgtatgacgataaagatgtgatgtgggcatttgctacccgttgtcgtccgggtacagatgaagttttttttgatgatgttcctggcttttggctgatcccgtatatgagtcatggtaatgccgaagcagtgaaaggtggtaaagttgttagtgatgcactgctgaccgcagaatataccaccggtaaagattgggaaagcgcagatttcaaaaacagctatccgaaacgtatccaggataaagttctgaatagctgggaacgcctgggtttcaaaaaactggattaataaggatccgaattcgagctcggcgcgcctgcaggtcgacaagcttgcggccgcataatgcttaagtcgaacagaaagtaatcgtattgtacacggccgcataatcgaaattaatacgactcactataggggaattgtgagcggataacaattccccatcttagtatattagttaagtataagaaggagatatacatatgaaacgactcattgtaggcatcagcggtgccagcggcgcgatttatggcgtgcgcttattacaggttctgcgcgatgtcacagatatcgaaacgcatctggtgatgagccaggcagcgcgccagaccttatccctcgaaacggatttttctctgcgcgaagtgcaggcattagccgatgtcacgcacgatgcgcgcgatattgccgccagcatctcttccggttctttccagacgctggggatggtgattttaccctgttcaatcaaaaccctttccggcattgtccatagctatactgatggcttactgacccgtgcggcagatgtggtgctgaaagagcgtcgcccgttggtgctctgcgtgcgtgaaacaccattgcacttaggccatctgcgtttaatgactcaggcggcagaaatcggtgcggtgattatgcctcccgttccggcgttttatcatcgcccgcaatcccttgatgatgtgataaatcagacggttaatcgtgttcttgaccagtttgcgataacccttcctgaagatctctttgcccgctggcagggcgcataataaggtaccgaaggagatatacatatgcaggttgatctgctgggtagcgcacagagcgcacatgcactgcacctgtttcatcagcatagtccgctggttcattgtatgaccaatgatgttgttcagacctttaccgcaaataccctgctggcactgggtgcaagtccggcaatggttattgaaaccgaagaagcaagccagtttgcagcaattgcaagcgcactgctgattaatgttggcaccctgacccagcctcgtgcacaggcaatgcgtgcagcagttgaacaggcaaaaagcagccagaccccgtggaccctggacccggttgcagttggtgcactggattatcgtcgtcatttttgtcatgaactgctgagctttaaaccggcagcaattcgtggtaatgcaagcgaaattatggcactggcaggtattgcaaatggtggtcgtggtgttgataccaccgatgcagcagcaaatgcaattccggcagcacagaccctggcacgtgaaaccggtgcaattgttgttgttaccggtgaaatggattatgttaccgatggtcatcgtattattggtattcatggtggtgatccgctgatgaccaaagttgttggcaccggttgtgcactgagcgcagttgttgcagcatgttgtgcactgcctggtgataccctggaaaatgttgcaagcgcatgtcattggatgaaacaggcaggcgaacgtgcagttgcacgtagcgaaggtccgggtagctttgttccgcattttctggatgcactgtggcagctgacccaggaagttcaggcataataattaattaacctaggctgctgccaccgctgagcaataactagcataaccccttggggcctctaaacgggtcttgaggggttttttgctgaaaggaggaactatatccggattggcgaatgggacgcgccctgtagcggcgcattaagcgcggcgggtgtggtggttacgcgcagcgtgaccgctacacttgccagcgccctagcgcccgctcctttcgctttcttcccttcctttctcgccacgttcgccggctttccccgtcaagctctaaatcgggggctccctttagggttccgatttagtgctttacggcacctcgaccccaaaaaacttgattagggtgatggttcacgtagtgggccatcgccctgatagacggtttttcgccctttgacgttggagtccacgttctttaatagtggactcttgttccaaactggaacaacactcaaccctatctcggtctattcttttgatttataagggattttgccgatttcggcctattggttaaaaaatgagctgatttaacaaaaatttaacgcgaattttaacaaaatattaacgtttacaatttctggcggcacgatggcatgagattatcaaaaaggatcttcacctagatccttttaaattaaaaatgaagttttaaatcaatctaaagtatatatgagtaaacttggtctgacagttaccaatgcttaatcagtgaggcacctatctcagcgatctgtctatttcgttcatccatagttgcctgactccccgtcgtgtagataactacgatacgggagggcttaccatctggccccagtgctgcaatgataccgcgagacccacgctcaccggctccagatttatcagcaataaaccagccagccggaagggccgagcgcagaagtggtcctgcaactttatccgcctccatccagtctattaattgttgccgggaagctagagtaagtagttcgccagttaatagtttgcgcaacgttgttgccattgctacaggcatcgtggtgtcacgctcgtcgtttggtatggcttcattcagctccggttcccaacgatcaaggcgagttacatgatcccccatgttgtgcaaaaaagcggttagctccttcggtcctccgatcgttgtcagaagtaagttggccgcagtgttatcactcatggttatggcagcactgcataattctcttactgtcatgccatccgtaagatgcttttctgtgactggtgagtactcaaccaagtcattctgagaatagtgtatgcggcgaccgagttgctcttgcccggcgtcaatacgggataataccgcgccacatagcagaactttaaaagtgctcatcattggaaaacgttcttcggggcgaaaactctcaaggatcttaccgctgttgagatccagttcgatgtaacccactcgtgcacccaactgatcttcagcatcttttactttcaccagcgtttctgggtgagcaaaaacaggaaggcaaaatgccgcaaaaaagggaataagggcgacacggaaatgttgaatactcatactcttcctttttcaatcatgattgaagcatttatcagggttattgtctcatgagcggatacatatttgaatgtatttagaaaaataaacaaataggtcatgaccaaaatcccttaacgtgagttttcgttccactgagcgtcagaccccgtagaaaagatcaaaggatcttcttgagatcctttttttctgcgcgtaatctgctgcttgcaaacaaaaaaaccaccgctaccagcggtggtttgtttgccggatcaagagctaccaactctttttccgaaggtaactggcttcagcagagcgcagataccaaatactgtccttctagtgtagccgtagttaggccaccacttcaagaactctgtagcaccgcctacatacctcgctctgctaatcctgttaccagtggctgctgccagtggcgataagtcgtgtcttaccgggttggactcaagacgatagttaccggataaggcgcagcggtcgggctgaacggggggttcgtgcacacagcccagcttggagcgaacgacctacaccgaactgagatacctacagcgtgagctatgagaaagcgccacgcttcccgaagggagaaaggcggacaggtatccggtaagcggcagggtcggaacaggagagcgcacgagggagcttccagggggaaacgcctggtatctttatagtcctgtcgggtttcgccacctctgacttgagcgtcgatttttgtgatgctcgtcaggggggcggagcctatggaaaaacgccagcaacgcggcctttttacggttcctggccttttgctggccttttgctcacatgttctttcctgcgttatcccctgattctgtggataaccgtattaccgcctttgagtgagctgataccgctcgccgcagccgaacgaccgagcgcagcgagtcagtgagcgaggaagcggaagagcgcctgatgcggtattttctccttacgcatctgtgcggtatttcacaccgcatatatggtgcactctcagtacaatctgctctgatgccgcatagttaagccagtatacactccgctatcgctacgtgactgggtcatggctgcgccccgacacccgccaacacccgctgacgcgccctgacgggcttgtctgctcccggcatccgcttacagacaagctgtgaccgtctccgggagctgcatgtgtcagaggttttcaccgtcatcaccgaaacgcgcgaggcagctgcggtaaagctcatcagcgtggtcgtgaagcgattcacagatgtctgcctgttcatccgcgtccagctcgttgagtttctccagaagcgttaatgtctggcttctgataaagcgggccatgttaagggcggttttttcctgtttggtcactgatgcctccgtgtaagggggatttctgttcatgggggtaatgataccgatgaaacgagagaggatgctcacgatacgggttactgatgatgaacatgcccggttactggaacgttgtgagggtaaacaactggcggtatggatgcggcgggaccagagaaaaatcactcagggtcaatgccagcgcttcgttaatacagatgtaggtgttccacagggtagccagcagcatcctgcgatgcagatccggaacataatggtgcagggcgctgacttccgcgtttccagactttacgaaacacggaaaccgaagaccattcatgttgttgctcaggtcgcagacgttttgcagcagcagtcgcttcacgttcgctcgcgtatcggtgattcattctgctaaccagtaaggcaaccccgccagcctagccgggtcctcaacgacaggagcacgatcatgctagtcatgccccgcgcccaccggaaggagctgactgggttgaaggctctcaagggcatcggtcgagatcccggtgcctaatgagtgagctaacttacattaattgcgttgcgctcactgcccgctttccagtcgggaaacctgtcgtgccagctgcattaatgaatcggccaacgcgcggggagaggcggtttgcgtattgggcgccagggtggtttttcttttcaccagtgagacgggcaacagctgattgcccttcaccgcctggccctgagagagttgcagcaagcggtccacgctggtttgccccagcaggcgaaaatcctgtttgatggtggttaacggcgggatataacatgagctgtcttcggtatcgtcgtatcccactaccgagatgtccgcaccaacgcgcagcccggactcggtaatggcgcgcattgcgcccagcgccatctgatcgttggcaaccagcatcgcagtgggaacgatgccctcattcagcatttgcatggtttgttgaaaaccggacatggcactccagtcgccttcccgttccgctatcggctgaatttgattgcgagtgagatatttatgccagccagccagacgcagacgcgccgagacagaacttaatgggcccgctaacagcgcgatttgctggtgacccaatgcgaccagatgctccacgcccagtcgcgtaccgtcttcatgggagaaaataatactgttgatgggtgtctggtcagagacatcaagaaataacgccggaacattagtgcaggcagcttccacagcaatggcatcctggtcatccagcggatagttaatgatcagcccactgacgcgttgcgcgagaagattgtgcaccgccgctttacaggcttcgacgccgcttcgttctaccatcgacaccaccacgctggcacccagttgatcggcgcgagatttaatcgccgcgacaatttgcgacggcgcgtgcagggccagactggaggtggcaacgccaatcagcaacgactgtttgcccgccagttgttgtgccacgcggttgggaatgtaattcagctccgccatcgccgcttccactttttcccgcgttttcgcagaaacgtggctggcctggttcaccacgcgggaaacggtctgataagagacaccggcatactctgcgacatcgtataacgttactggtttcacattcaccaccctgaattgactctcttccgggcgctatcatgccataccgcgaaaggttttgcgccattcgatggtgtccgggatctcgacgctctcccttatgcgactcctgcattaggaagcagcccagtagtaggttgaggccgttgag

SEQ ID NO: 39 - protein, 209 aa, Escherichia coli
  nudF Escherichia coli (strain K12)
MLKPDNLPVTFGKNDVEIIARETLYRGFFSLDLYRFRHRLFNGQMSHEVRREIFERGHAAVLLPFDPVRDEVVLIEQIRIAAYDTSETPWLLEMVAGMIEEGESVEDVARREAIEEAGLIVKRTKPVLSFLASPGGTSERSSIMVGEVDATTASGIHGLADENEDIRVHVVSREQAYQWVEEGKIDNAASVIALQWLQLHHQALKNEWA

SEQ ID NO: 40 - protein, 129 aa, Escherichia coli
  mutT Escherichia coli (strain K12)
MKKLQIAVGIIRNENNEIFITRRAADAHMANKLEFPGGKIEMGETPEQAVVRELQEEVGITPQHFSLFEKLEYEFPDRHITLWFWLVERWEGEPWGKEGQPGEWMSLVGLNADDFPPANEPVIAKLKRL

SEQ ID NO: 41 - protein, 280 aa, Escherichia coli
  apaH Escherichia coli (strain K12)
MATYLIGDVHGCYDELIALLHKVEFTPGKDTLWLTGDLVARGPGSLDVLRYVKSLGDSVRLVLGNHDLHLLAVFAGISRNKPKDRLTPLLEAPDADELLNWLRRQPLLQIDEEKKLVMAHAGITPQWDLQTAKECARDVEAVLSSDSYPFFLDAMYGDMPNNWSPELRGLGRLRFITNAFTRMRFCFPNGQLDMYSKESPEEAPAPLKPWFAIPGPVAEEYSIAFGHWASLEGKGTPEGIYALDTGCCWGGTLTCLRWEDKQYFVQPSNRHKDLGEAAAS

SEQ ID NO: 42 - protein, 550 aa, Escherichia coli
  ushA Escherichia coli (strain K12)
MKLLQRGVALALLTTFTLASETALAYEQDKTYKITVLHTNDHHGHFWRNEYGEYGLAAQKTLVDGIRKEVAAEGGSVLLLSGGDINTGVPESDLQDAEPDFRGMNLVGYDAMAIGNHEFDNPLTVLRQQEKWAKFPLLSANIYQKSTGERLFKPWALFKRQDLKIAVIGLTTDDTAKIGNPEYFTDIEFRKPADEAKLVIQELQQTEKPDIIIAATHMGHYDNGEHGSNAPGDVEMARALPAGSLAMIVGGHSQDPVCMAAENKKQVDYVPGTPCKPDQQNGIWIVQAHEWGKYVGRADFEFRNGEMKMVNYQLIPVNLKKKVTWEDGKSERVLYTPEIAENQQMISLLSPFQNKGKAQLEVKIGETNGRLEGDRDKVRFVQTNMGRLILAAQMDRTGADFAVMSGGGIRDSIEAGDISYKNVLKVQPFGNVVVYADMTGKEVIDYLTAVAQMKPDSGAYPQFANVSFVAKDGKLNDLKIKGEPVDPAKTYRMATLNFNATGGDGYPRLDNKPGYVNTGFIDAEVLKAYIQKSSPLDVSVYEPKGEVSWQ

SEQ ID NO: 43 - protein, 513 aa, Escherichia coli
  ppX Escherichia coli (strain K12)
MPIHDKSPRPQEFAAVDLGSNSFHMVIARVVDGAMQIIGRLKQRVHLADGLGPDNMLSEEAMTRGLNCLSLFAERLQGFSPASVCIVGTHTLRQALNATDFLKRAEKVIPYPIEIISGNEEARLIFMGVEHTQPEKGRKLVIDIGGGSTELVIGENFEPILVESRRMGCVSFAQLYFPGGVINKENFQRARMAAAQKLETLTWQFRIQGWNVAMGASGTIKAAHEVLMEMGEKDGIITPERLEKLVKEVLRHRNFASLSLPGLSEERKTVFVPGLAILCGVFDALAIRELRLSDGALREGVLYEMEGRFRHQDVRSRTASSLANQYHIDSEQARRVLDTTMQMYEQWREQQPKLAHPQLEALLRWAAMLHEVGLNINHSGLHRHSAYILQNSDLPGFNQEQQLMMATLVRYHRKAIKLDDLPRFTLFKKKQFLPLIQLLRLGVLLNNQRQATTTPPTLTLITDDSHWTLRFPHDWFSQNALVLLDLEKEQEYWEGVAGWRLKIEEESTPEIAA

SEQ ID NO: 44 - protein, 494 aa, Escherichia coli
  gppA Escherichia coli (strain K12)
MGSTSSLYAAIDLGSNSFHMLVVREVAGSIQTLTRIKRKVRLAAGLNSENALSNEAMERGWQCLRLFAERLQDIPPSQIRVVATATLRLAVNAGDFIAKAQEILGCPVQVISGEEEARLIYQGVAHTTGGADQRLVVDIGGASTELVTGTGAQTTSLFSLSMGCVTWLERYFADRNLGQENFDAAEKAAREVLRPVADELRYHGWKVCVGASGTVQALQEIMMAQGMDERITLEKLQQLKQRAIHCGRLEELEIDGLTLERALVFPSGLAILIAIFTELNIQCMTLAGGALREGLVYGMLHLAVEQDIRSRTLRNIQRRFMIDIDQAQRVAKVAANFFDQVENEWHLEAISRDLLISACQLHEIGLSVDFKQAPQHAAYLVRNLDLPGFTPAQKKLLATLLLNQTNPVDLSSLHQQNAVPPRVAEQLCRLLRLAIIFASRRRDDLVPEMTLQANHELLTLTLPQGWLTQHPLGKEIIAQESQWQSYVHWPLEVH

SEQ ID NO: 45 - protein, 257 aa, Escherichia coli
  nudC Escherichia coli (strain K12)
MDRIIEKLDHGWWVVSHEQKLWLPKGELPYGEAANFDLVGQRALQIGEWQGEPVWLVQQQRRHDMGSVRQVIDLDVGLFQLAGRGVQLAEFYRSHKYCGYCGHEMYPSKTEWAMLCSHCRERYYPQIAPCIIVAIRRDDSILLAQHTRHRNGVHTVLAGFVEVGETLEQAVAREVMEESGIKVKNLRYVTSQPWPFPQSLMTAFMAEYDSGDIVIDPKELLEANWYRYDDLPLLPPPGTVARRLIEDTVAMCRAEYE

SEQ ID NO: 46 - protein, 197 aa, Escherichia coli
  yhdE Escherichia coli (strain K12)
MTSLYLASGSPRRQELLAQLGVTFERIVTGIEEQRQPQESAQQYVVRLAREKARAGVAQTAKDLPVLGADTIVILNGEVLEKPRDAEHAAQMLRKLSGQTHQVMTAVALADSQHILDCLVVTDVTFRTLTDEDIAGYVASDEPLDKAGAYGIQGLGGCFVRKINGSYHAVVGLPLVETYELLSNFNALREKRDKHDG

SEQ ID NO: 47 - protein, 246 aa, Escherichia coli
  cysQ Escherichia coli (strain K12)
MLDQVCQLARNAGDAIMQVYDGTKPMDVVSKADNSPVTAADIAAHTVIMDGLRTLTPDVPVLSEEDPPGWEVRQHWQRYWLVDPLDGTKEFIKRNGEFTVNIALIDHGKPILGVVYAPVMNVMYSAAEGKAWKEECGVRKQIQVRDARPPLVVISRSHADAELKEYLQQLGEHQTTSIGSSLKFCLVAEGQAQLYPRFGPTNIWDTAAGHAVAAAAGAHVHDWQGKPLDYTPRESFLNPGFRVSIY

SEQ ID NO: 48 - protein, 238 aa, Escherichia coli
  yigB Escherichia coli (strain K12)
MRFYRPLGRISALTFDLDDTLYDNRPVILRTEREALTFVQNYHPALRSFQNEDLQRLRQAVREAEPEIYHDVTRWRFRSIEQAMLDAGLSAEEASAGAHAAMINFAKWRSRIDVPQQTHDTLKQLAKKWPLVAITNGNAQPELFGLGDYFEFVLRAGPHGRSKPFSDMYFLAAEKLNVPIGEILHVGDDLTTDVGGAIRSGMQACWIRPENGDLMQTWDSRLLPHLEISRLASLTSLI

SEQ ID NO: 49 - protein, 271 aa, Escherichia coli
  ybjl Escherichia coli (strain K12)
MSIKLIAVDMDGTFLSDQKTYNRERFMAQYQQMKAQGIRFVVASGNQYYQLISFFPEIANEIAFVAENGGWVVSEGKDVFNGELSKDAFATVVEHLLTRPEVEIIACGKNSAYTLKKYDDAMKTVAEMYYHRLEYVDNFDNLEDIFFKFGLNLSDELIPQVQKALHEAIGDIMVSVHTGNGSIDLIIPGVHKANGLRQLQKLWGIDDSEVVVFGDGGNDIEMLRQAGFSFAMENAGSAVVAAAKYRAGSNNREGVLDVIDKVLKHEAPFDQ

SEQ ID NO: 50 - protein, 332 aa, Escherichia coli
  fbp Escherichia coli (strain K12)
MKTLGEFIVEKQHEFSHATGELTALLSAIKLGAKIIHRDINKAGLVDILGASGAENVQGEVQQKLDLFANEKLKAALKARDIVAGIASEEEDEIVVFEGCEHAKYVVLMDPLDGSSNIDVNVSVGTIFSIYRRVTPVGTPVTEEDFLQPGNKQVAAGYVVYGSSTMLVYTTGCGVHAFTYDPSLGVFCLCQERMRFPEKGKTYSINEGNYIKFPNGVKKYIKFCQEEDKSTNRPYTSRYIGSLVADFHRNLLKGGIYLYPSTASHPDGKLRLLYECNPMAFLAEQAGGKASDGKERILDIIPETLHQRRSFFVGNDHMVEDVERFIREFPDA

SEQ ID NO: 51 - protein, 248 aa, Haloferax volcanii
  Haloferax volcanii (strain ATCC 29605 / DSM 3757 / JCM 8879 / NBRC 14742 / NCIMB 2012 / VKM B-1768 / DS2)
MSLVVLKLGGSVVTDKDEPETVDEAGLAAAADAVAPLAESRRVVVVHGGGSFGHHHAAEHGVSSESGSHDARGVRAIHDAMKRLNDAVLDALEERGVAALPVHPLSAGAREADGSLSLPLAATETMLDEGFVPVLHGDVISHAGKGATIVSGDDLVVSLASGLGADRVGLCSTVPGVLDADGDVIPEITAFADAADALGGSDSTDVTGGMAAKVRKLLALGAPAHVFGPEGLSAFVAGESPGTVIRGE

SEQ ID NO: 52 - protein, 266 aa, Methanothermobacter thermautotrophicus
  Methanothermobacter thermautotrophicus (strain ATCC 29096 / DSM 1053 / JCM 10044 / NBRC 100330 / Delta H)
MIILKLGGSVITRKDSEEPAIDRDNLERIASEIGNASPSSLMIVHGAGSFGHPFAGEYRIGSEIENEEDLRRRRFGFALTQNWVKKLNSHVCDALLAEGIPAVSMQPSAFIRAHAGRISHADISLIRSYLEEGMVPVVYGDVVLDSDRRLKFSVISGDQLINHFSLRLMPERVILGTDVDGVYTRNPKKHPDARLLDVIGSLDDLESLDGTLNTDVTGGMVGKIRELLLLAEKGVESEIINAAVPGNIERALLGEEVRGTRITGKH

SEQ ID NO: 53 - protein, 260 aa, Methanocaldococcus jannaschii
  Methanocaldococcus jannaschii (strain ATCC 43067 / DSM 2661 / JAL-1 / JCM 10045 / NBRC 100440)
MLTILKLGGSILSDKNVPYSIKWDNLERIAMEIKNALDYYKNQNKEIKLILVHGGGAFGHPVAKKYLKIEDGKKIFINMEKGFWEIQRAMRRFNNIIIDTLQSYDIPAVSIQPSSFVVFGDKLIFDTSAIKEMLKRNLVPVIHGDIVIDDKNGYRIISGDDIVPYLANELKADLILYATDVDGVLIDNKPIKRIDKNNIYKILNYLSGSNSIDVTGGMKYKIDMIRKNKCRGFVFNGNKANNIYKALLGEVEGTEIDFSE

SEQ ID NO: 54 - protein, 245 aa, Thermoplasma acidophilum
  Thermoplasma acidophilum (strain ATCC 25905 / DSM 1728 / JCM 9062 / NBRC 15155 / AMRC-C165)
MMILKIGGSVITDKSAYRTARTYAIRSIVKVLSGIEDLVCVVHGGGSFGHIKAMEFGLPGPKNPRSSIGYSIVHRDMENLDLMVIDAMIEMGMRPISVPISALRYDGRFDYTPLIRYIDAGFVPVSYGDVYIKDEHSYGIYSGDDIMADMAELLKPDVAVFLTDVDGIYSKDPKRNPDAVLLRDIDTNITFDRVQNDVTGGIGKKFESMVKMKSSVKNGVYLINGNHPERIGDIGKESFIGTVIR

SEQ ID NO: 55 - protein, 471 aa, Escherichia coli
  phoA Escherichia coli (strain K12)
MKQSTIALALLPLLFTPVTKARTPEMPVLENRAAQGDITAPGGARRLTGDQTAALRDSLSDKPAKNIILLIGDGMGDSEITAARNYAEGAGGFFKGIDALPLTGQYTHYALNKKTGKPDYVTDSAASATAWSTGVKTYNGALGVDIHEKDHPTILEMAKAAGLATGNVSTAELQDATPAALVAHVTSRKCYGPSATSEKCPGNALEKGGKGSITEQLLNARADVTLGGGAKTFAETATAGEWQGKTLREQAQARGYQLVSDAASLNSVTEANQQKPLLGLFADGNMPVRWLGPKATYHGNIDKPAVTCTPNPQRNDSVPTLAQMTDKAIELLSKNEKGFFLQVEGASIDKQDHAANPCGQIGETVDLDEAVQRALEFAKKEGNTLVIVTADHAHASQIVAPDTKAPGLTQALNTKDGAVMVMSYGNSEEDSQEHTGSQLRIAAYGPHAANVVGLTDQTDLFYTMKAALGLK

SEQ ID NO: 56 - protein, 271 aa, Escherichia coli
  ybiV Escherichia coli (strain K12)
MSVKVIVTDMDGTFLNDAKTYNQPRFMAQYQELKKRGIKFVVASGNQYYQLISFFPELKDEISFVAENGALVYEHGKQLFHGELTRHESRIVIGELLKDKQLNFVACGLQSAYVSENAPEAFVALMAKHYHRLKPVKDYQEIDDVLFKFSLNLPDEQIPLVIDKLHVALDGIMKPVTSGFGFIDLIIPGLHKANGISRLLKRWDLSPQNVVAIGDSGNDAEMLKMARYSFAMGNAAENIKQIARYATDDNNHEGALNVIQAVLDNTSPFNS

SEQ ID NO: 57 - protein, 270 aa, Escherichia coli
  yidA Escherichia coli (strain K12)
MAIKLIAIDMDGTLLLPDHTISPAVKNAIAAARARGVNVVLTTGRPYAGVHNYLKELHMEQPGDYCITYNGALVQKAADGSTVAQTALSYDDYRFLEKLSREVGSHFHALDRTTLYTANRDISYYTVHESFVATIPLVFCEAEKMDPNTQFLKVMMIDEPAILDQAIARIPQEVKEKYTVLKSAPYFLEILDKRVNKGTGVKSLADVLGIKPEEIMAIGDQENDIAMIEYAGVGVAMDNAIPSVKEVANFVTKSNLEDGVAFAIEKYVLN

SEQ ID NO: 58 - protein, 172 aa, Escherichia coli
  pgpA Escherichia coli (strain K12)
MTILPRHKDVAKSRLKMSNPWHLLAVGFGSGLSPIVPGTMGSLAAIPFWYLMTFLPWQLYSLVVMLGICIGVYLCHQTAKDMGVHDHGSIVWDEFIGMWITLMALPTNDWQWVAAGFVIFRILDMWKPWPIRWFDRNVHGGMGIMIDDIVAGVISAGILYFIGHHWPLGILS

SEQ ID NO: 59 - protein, 211 aa, Escherichia coli [sequence omitted]

SEQ ID NO: 60 - protein, 254 aa, Escherichia coli
  pgpB Escherichia coli (strain K12)
MRSIARRTAVGAALLLVMPVAVWISGWRWQPGEQSWLLKAAFWVTETVTQPWGVITHLILFGWFLWCLRFRIKAAFVLFAILAAAILVGQGVKSWIKDKVQEPRPFVIWLEKTHHIPVDEFYTLKRAERGNLVKEQLAEEKNIPQYLRSHWQKETGFAFPSGHTMFAASWALLAVGLLWPRRRTLTIAILLVWATGVMGSRLLLGMHWPRDLVVATLISWALVAVATWLAQRICGPLTPPAEENREIAQREQES

SEQ ID NO: 61 - protein, 322 aa, Escherichia coli [sequence omitted]

SEQ ID NO: 62 - protein, 252 aa, Escherichia coli
  gph Escherichia coli (strain K12)
MNKFEDIRGVAFDLDGTLVDSAPGLAAAVDMALYALELPVAGEERVITWIGNGADVLMERALTWARQERATQRKTMGKPPVDDDIPAEEQVRILRKLFDRYYGEVAEEGTFLFPHVADTLGALQAKGLPLGLVTNKPTPFVAPLLEALDIAKYFSVVIGGDDVQNKKPHPDPLLLVAERMGIAPQQMLFVGDSRNDIQAAKAAGCPSVGLTYGYNYGEAIDLSQPDVIYQSINDLLPALGLPHSENQESKND

SEQ ID NO: 63 - protein, 225 aa, Escherichia coli
  yjjG Escherichia coli (strain K12)
MKWDWIFFDADETLFTFDSFTGLQRMFLDYSVTFTAEDFQDYQAVNKPLWVDYQNGAITSLQLQHGRFESWAERLNVEPGKLNEAFINAMAEICTPLPGAVSLLNAIRGNAKIGIITNGFSALQQVRLERTGLRDYFDLLVISEEVGVAKPNKKIFDYALEQAGNPDRSRVLMVGDTAESDILGGINAGLATCWLNAHHREQPEGIAPTWTVSSLHELEQLLCKH

SEQ ID NO: 64 - protein, 266 aa, Escherichia coli
  yjgL Escherichia coli (strain K12)
MYQVVASDLDGTLLSPDHTLSPYAKETLKLLTARGINFVFATGRHHVDVGQIRDNLEIKSYMITSNGARVHDLDGNLIFAHNLDRDIASDLFGVVNDNPDIITNVYRDDEWFMNRHRPEEMRFFKEAVFQYALYEPGLLEPEGVSKVFFTCDSHEQLLPLEQAINARWGDRVNVSFSTLTCLEVMAGGVSKGHALEAVAKKLGYSLKDCIAFGDGMNDAEMLSMAGKGCIMGSAHQRLKDLHPELEVIGTNADDAVPHYLRKLYLS

SEQ ID NO: 65 - protein, 550 aa, Escherichia coli; identical to SEQ ID NO: 42
  ushA Escherichia coli (strain K12)

SEQ ID NO: 66 - protein, 197 aa, Escherichia coli
  UbiX-like flavin prenyltransferase from Escherichia coli O157:H7
MKLIVGMTGATGAPLGVALLQALREMPNVETHLVMSKWAKTTIELETPYSARDVAALADFSHNPADQAATISSGSFRTDGMIVIPCSMKTLAGIRAGYADGLVGRAADVVLKEGRKLVLVPREMPLSTIHLENMLALSRMGVAMVPPMPAFYNHPETVDDIVHHVVARVLDQFGLEHPHARRWQGLPQARNFSQENE

SEQ ID NO: 67 - protein, 92 aa, Escherichia coli (strain K12)
MSKVCIIAWVYGRVQGVGFRYTTQYEAKRLGLTGYAKNLDDGSVEVVACGEEGQVEKLMQWLKSGGPRSARVERVLSEPHHPSGELTDFRIR

SEQ ID NO: 68 - protein, 862 aa, Saccharomyces cerevisiae (strain ATCC 204508 / S288 c)
MQYVGRALGSVSKTWSSINPATLSGAIDVIVVEHPDGRLSCSPFHVRFGKFQILKPSQKKVQVFINEKLSNMPMKLSDSGEAYFVFEMGDQVTDVPDELLVSPVMSATSSPPQSPETSILEGGTEGEGEGENENKKKEKKVLEEPDFLDINDTGDSGSKNSETTGSLSPTESSTTTPPDSVEERKLVEQRTKNFQQKLNKKLTEIHIPSKLDNNGDLLLDTEGYKPNKNMMHDTDIQLKQLLKDEFGNDSDISSFIKEDKNGNIKIVNPYEHLTDLSPPGTPPTMATSGSVLGLDAMESGSTLNSLSSSPSGSDTEDETSFSKEQSSKSEKTSKKGTAGSGETEKRYIRTIRLTNDQLKCLNLTYGENDLKFSVDHGKAIVTSKLFVWRWDVPIVISDIDGTITKSDALGHVLAMIGKDWTHLGVAKLFSEISRNGYNILYLTARSAGQADSTRSYLRSIEQNGSKLPNGPVILSPDRTMAALRREVILKKPEVFKIACLNDIRSLYFEDSDNEVDTEEKSTPFFAGFGNRITDALSYRTVGIPSSRIFTINTEGEVHMELLELAGYRSSYIHINELVDHFFPPVSLDSVDLRTNTSMVPGSPPNRTLDNFDSEITSGRKTLFRGNQEEKFTDVNFWRDPLVDIDNLSDISNDDSDNIDEDTDVSQQSNISRNRANSVKTAKVTKAPQRNVSGSTNNNEVLAASSDVENASDLVSSHSSSGSTPNKSTMSKGDIGKQIYLELGSPLASPKLRYLDDMDDEDSNYNRTKSRRASSAAATSIDKEFKKLSVSKAGAPTRIVSKINVSNDVHSLGNSDTESRREQSVNETGRNQLPHNSMDDKDLDSRVSDEFDDDEFDEDEFED

SEQ ID NO: 69 - protein, 132 aa, Methanocaldococcus jannaschii (strain ATCC 43067 / DSM 2661 / JAL-1 /JCM 10045 / NBRC 100400)
MIIEGEVVSGLGEGRYFLSLPPYKEIFKKILGFEPYEGTLNLKLDREFDINKFKYIETEDFEFNGKRFFGVKVLPIKILIGNKKIDGAIVVPKKTYHSSEIIEIIAPMKLREQFNLKDGDVIKILIKGDKDE

SEQ ID NO: 70 - protein, 197 aa, Klebsiella pneumoniae
  UbiX-like flavin prenyltransferase from Klebsiella pneumoniae
MKLIIGMTGATGAPLGVALLQALRDMPEVETHLVMSKWAKTTIELETPWTAREVAALADFSHSPADQAATISSGSFRTDGMIVIPCSMKTLAGIRAGYAEGLVGRAADVVLKEGRKLVLVPREMPLSTIHLENMLALSRMGVAMVPPMPAYYNHPETVDDITNHIVTRVLDQFGLDYHKARRWNGLRTAEQFAQEIE

SEQ ID NO: 71 - protein, 221 aa, Hypocrea atroviridis (strain ATCC 20476 / IMI 206040)
  Flavin prenyltransferase PAD1, mitochondrial from Hypocrea atroviridis (strain ATCC 20476 / IMI 206040)
MSPSLTDEESLAISHANGSNGTAPYQPPQPRRKRIIVAMTGATGTILGIKLLIALRRLNVETHLVISKWAEQTLKYETDYHPSNVRALADHVYGINDMAAAISSGSFRVDGMIVVPCSMKTLAGITTGLCDDLISRAADVMLKERRKLVLVARETPLSEIHLRNMLDVTRAGAIIFPPVPAYYIRPASVDDLVNQSVGRMLDLFDLDTEEFERWNGWKKDN